European Patent Application EP 4 115 898 A1, published January 11, 2023. Title: Use of snake NGF and preproNGF for the treatment of Alzheimer's Disease. Applicant: Qi, Zhankai. Application PCT/001. The sequence listing filed with the application follows.

SEQUENCE LISTING (8 sequences)

SEQ ID NO: 1 - protein, 241 aa, 噬鱼蝮（Agkistrodon piscivorus）
MSMLCYTLIIAFLIGIWAAPKSEDNVPLGSPATSDLSDTSCAKTHEALKTSRNTDQHYPAPKKAEDQEFGSAANIIVDPKLFQKRRFQSPRVLFSTQPPPLSRDEQNVDNANSLNRNIRAKREDHPVHNRGEYSVCDSVNVWVANKTTATDIRGNVVTVMVDVNINNNVYKQYFFETKCRNPNPVPTGCRGIDARHWNSYCTTTNTFVKALTMEGNQASWRFIRIDSACVCVISRKNENFG

SEQ ID NO: 2 - protein, 110 aa, 噬鱼蝮（Agkistrodon piscivorus）
HNRGEYSVCDSVNVWVANKTTATDIRGNVVTVMVDVNINNNVYKQYFFETKCRNPNPVPTGCRGIDARHWNSYCTTTNTFVKALTMEGNQASWRFIRIDSACVCVISRKN

SEQ ID NO: 3 - protein, 221 aa, 噬鱼蝮（Agkistrodon piscivorus）
SCMKAAPMKEVSIRGQGSLAYPGLRTQGNLETLSGPNDATRGLTSLADTFEHVIEELLDEQQAIQPSKENKDADLYSSRVMLSSQVPLEPPLLFLLEEYKNYLDAANMSMRVRRHSDPARRGELSVCDSTSEWVTAAEKKTAVDMSGATVTVLEKVPVPKGQLKQYFYETKCSTKGYAKEGCRGIDKRYWNSQCRTTQSYVRALTMDNKKRVGWRFIRIDT

SEQ ID NO: 4 - protein, 103 aa, 噬鱼蝮（Agkistrodon piscivorus）
ARRGELSVCDSTSEWVTAAEKKTAVDMSGATVTVLEKVPVPKGQLKQYFYETKCSAKGYAKEGCRGIDKRYWNSQCRTTQSYVRALTMDNKKRVGWRFIRIDT

SEQ ID NO: 5 - protein, 241 aa, 原矛头蝮（Protobothrops mucrosquamatus）
MSMLCYTLIIAFLIGIWAAPKSEDNVPLGSPATSDLSDTSCAKTHEALKTSRNTDHHYPAPKKAEDQEFGSAANIIVDPKLFQKRRFQSPRVLFSTQPPPLSRDEQSVDNANSLNRNIRAKREDHPVHNRGEYSVCDSVNVWVANKTTATDIRGNLVTVMVDVNLNNNVYKQYFFETKCRNPNPVPTGCRGIDSRHWNSYCTTTHTFVKALTMEGKQASWRFIRIDAACVCVISRKNENFG

SEQ ID NO: 6 - protein, 110 aa, 原矛头蝮（Protobothrops mucrosquamatus）
HNRGEYSVCDSVNVWVANKTTATDIRGNLVTVMVDVNLNNNVYKQYFFETKCRNPNPVPTGCRGIDSRHWNSYCTTTHTFVKALTMEGKQASWRFIRIDAACVCVISRKN

SEQ ID NO: 7 - protein, 244 aa, 钝鼻蝰(Macrovipera lebetina)
MSMLCYTLIIAFLIGIWAAPKSEDNVSLGSPATPDLSDTSCAKTHEALKTSRNTDQHYPAPKKAEDQEFGSAANIIVDPKLFQKRRFQSPRVLFSTQPPPLSRDEQSVEFLDNADSLNRNIRAKRATHPVHNRGEFSVCDSVSVWVANKTTATDIRGNVVTVMVDVKLNNNVYRQYFFETKCKNPSPVSSGCRGIDAKHWNSYCTTTDTFVRALTMEGNQASWRFIRIDTACVCVISRKNDNFG

SEQ ID NO: 8 - protein, 110 aa, 钝鼻蝰(Macrovipera lebetina)
HNRGEFSVCDSVSVWVANKTTATDIRGNVVTVMVDVKLNNNVYRQYFFETKCKNPSPVSSGCRGIDAKHWNSYCTTTDTFVRALTMEGNQASWRFIRIDTACVCVISRKN